European Patent Specification EP 3 528 787 B1, published January 7, 2026. Title: Pharmaceutical Formulations and Methods of Making the Same. Applicant: AMGEN INC. GOSS, Monica BALL, Nicole. Application XX/XXX,XXX. The sequence listing filed with the application follows.

SEQUENCE LISTING (1 sequence)

SEQ ID NO: 1 - protein, 469 aa, Chinese hamster ovarian cell
LPALAQVAFTRYAPEPGSTCRLREYYDQTAQMCCSKCSPGQHAKVFCTKTSDTVCDSCEDSTYTQLWNWVRECLSCGSRCSSDQVETQACTREQNRICTCRPGWYCALSKQEGCRLCAPLRKCRPGFGVARPGTETSDVVCKPCAPGTFSNTTSSTDICRPHQICNVVAIPGNASMDAVCTSTSPTRSMAPGAVHLPQPVSTRSQHTQPTPEPSTAPSTSFLLPMGPSPPAEGSTGDEPKSCDKTHTCPPCPAPELLGGPSVFLFPPKPKDTLMISRTPEVTCVVVDVSHEDPEVKFNWYVDGVEVHNAKTKPREEQYNSTYRVVSVLTVLHQDWLNGKEYKCKVSNKALPAPIEKTISKAKGQPREPQVYTLPPSREEMTKNQVSLTCLVKGFYPSDIAVEWESNGQPENNYKTTPPVLDSDGSFFLYSKLTVDKSRWQQGNVFSCSVMHEALHNHYTQKSLSLSPGK